European Patent Specification EP 3 518 972 B1, published December 25, 2024. Title: ANTIGEN BINDING MOLECULES AND METHODS OF USE THEREOF. Applicant: KITE PHARMA, INC. The sequence listing filed with the application follows.

SEQUENCE LISTING (82 sequences)

SEQ ID NO: 1 - protein, 267 aa, Artificial Sequence
  Description of Artificial Sequence: Synthetic polypeptide
MLLLVTSLLLCELPHPAFLLIPDIQMTQTTSSLSASLGDRVTISCRASQDISKYLNWYQQKPDGTVKLLIYHTSRLHSGVPSRFSGSGSGTDYSLTISNLEQEDIATYFCQQGNTLPYTFGGGTKLEITGSTSGSGKPGSGEGSTKGEVKLQESGPGLVAPSQSLSVTCTVSGVSLPDYGVSWIRQPPRKGLEWLGVIWGSETTYYNSALKSRLTIIKDNSKSQVFLKMNSLQTDDTAIYYCAKHYYYGGSYAMDYWGQGTSVTVSS

SEQ ID NO: 2 - DNA, 396 bp, Artificial Sequence
  Description of Artificial Sequence: Synthetic polynucleotide
atggagactgggctgcgctggcttctcctggtcgctgtgctcaaaggtgtccagtgtcaggagcagctggaggagtccgggggagacctggtcaagcctggaggaaccctgacagtcacctgcaaagcctctggattctccttcagtaacaatggaatttgctgggtccgccaggctccagggaaggggctggagtggatcggatgtctttatgttggtagtagtgataccacttactacgcgagctgggcgaaaggccgattcaccatctccaaaagctcgtcgaccacggtgactctacaaatgaccagtctgacagtcgcggacacggccacctatttctgtacgataaatctcggcttgtggggccccggcaccctggtcaccgtctcctca

SEQ ID NO: 3 - protein, 132 aa, Artificial Sequence
  Description of Artificial Sequence: Synthetic polypeptide
METGLRWLLLVAVLKGVQCQEQLEESGGDLVKPGGTLTVTCKASGFSFSNNGICWVRQAPGKGLEWIGCLYVGSSDTTYYASWAKGRFTISKSSSTTVTLQMTSLTVADTATYFCTINLGLWGPGTLVTVSS

SEQ ID NO: 4 - protein, 455 aa, Artificial Sequence
  Description of Artificial Sequence: Synthetic polypeptide
METGLRWLLLVAVLKGVQCQEQLEESGGDLVKPGGTLTVTCKASGFSFSNNGICWVRQAPGKGLEWIGCLYVGSSDTTYYASWAKGRFTISKSSSTTVTLQMTSLTVADTATYFCTINLGLWGPGTLVTVSSGQPKAPSVFPLAPCCGDTPSSTVTLGCLVKGYLPEPVTVTWNSGTLTNGVRTFPSVRQSSGLYSLSSVVSVTSSSQPVTCNVAHPATNTKVDKTVAPSTCSKPTCPPPELLGGPSVFIFPPKPKDTLMISRTPEVTCVVVDVSQDDPEVQFTWYINNEQVRTARPPLREQQFNSTIRVVSTLPIAHQDWLRGKEFKCKVHNKALPAPIEKTISKARGQPLEPKVYTMGPPREELSSRSVSLTCMINGFYPSDISVEWEKNGKAEDNYKTTPAVLDSDGSYFLYSKLSVPTSEWQRGDVFTCSVMHEALHNHYTQKSISRSPGK

SEQ ID NO: 5 - protein, 7 aa, Artificial Sequence
  Description of Artificial Sequence: Synthetic peptide
GFSFSNN

SEQ ID NO: 6 - protein, 6 aa, Artificial Sequence
  Description of Artificial Sequence: Synthetic peptide
YVGSSD

SEQ ID NO: 7 - protein, 4 aa, Artificial Sequence
  Description of Artificial Sequence: Synthetic peptide
NLGL

SEQ ID NO: 8 - DNA, 402 bp, Artificial Sequence
  Description of Artificial Sequence: Synthetic polynucleotide
atggacacgagggcccccactcagctgctggggctcctgctgctctggctcccaggtgccacatttgccatcgtggtgacccagactccatcttccaagtctgtccctgtgggaggcacagtcaccatcaattgccaggccagtgagagtgtttataatagcgactggttagcctggtatcagcagaaaccagggcagcctcccaagcaactgatctatgctgcatccactctggcatctggggtcccatcgcgcttcaaaggcagtggatctgggacacagttcactctcaccatcagcgatgtggtgtgtgacgatgctgccacttattattgtgcaggatataaaagtagtagtactgatgggattgctttcggcggagggaccgaggtggtggtcaaa

SEQ ID NO: 9 - protein, 134 aa, Artificial Sequence
  Description of Artificial Sequence: Synthetic polypeptide
MDTRAPTQLLGLLLLWLPGATFAIVVTQTPSSKSVPVGGTVTINCQASESVYNSDWLAWYQQKPGQPPKQLIYAASTLASGVPSRFKGSGSGTQFTLTISDVVCDDAATYYCAGYKSSSTDGIAFGGGTEVVVK

SEQ ID NO: 10 - protein, 238 aa, Artificial Sequence
  Description of Artificial Sequence: Synthetic polypeptide
MDTRAPTQLLGLLLLWLPGATFAIVVTQTPSSKSVPVGGTVTINCQASESVYNSDWLAWYQQKPGQPPKQLIYAASTLASGVPSRFKGSGSGTQFTLTISDVVCDDAATYYCAGYKSSSTDGIAFGGGTEVVVKGDPVAPTVLIFPPAADQVATGTVTIVCVANKYFPDVTVTWEVDGTTQTTGIENSKTPQNSADCTYNLSSTLTLTSTQYNSHKEYTCKVTQGTTSVVQSFNRGDC

SEQ ID NO: 11 - protein, 13 aa, Artificial Sequence
  Description of Artificial Sequence: Synthetic peptide
QASESVYNSDWLA

SEQ ID NO: 12 - protein, 7 aa, Artificial Sequence
  Description of Artificial Sequence: Synthetic peptide
AASTLAS

SEQ ID NO: 13 - protein, 12 aa, Artificial Sequence
  Description of Artificial Sequence: Synthetic peptide
AGYKSSSTDGIA

SEQ ID NO: 14 - DNA, 396 bp, Artificial Sequence; identical to SEQ ID NO: 2
  Description of Artificial Sequence: Synthetic polynucleotide

SEQ ID NO: 15 - protein, 132 aa, Artificial Sequence; identical to SEQ ID NO: 3
  Description of Artificial Sequence: Synthetic polypeptide

SEQ ID NO: 16 - protein, 455 aa, Artificial Sequence; identical to SEQ ID NO: 4
  Description of Artificial Sequence: Synthetic polypeptide

SEQ ID NO: 17 - DNA, 401 bp, Artificial Sequence
  Description of Artificial Sequence: Synthetic polynucleotide
atggacacgagggcccccactcagctgctggggctcctgctgctctggctcccaggtgccacacttgccatcgtggtgacccagactccatcttccaagtctgtccctgtgggaggcacagtcaccatcaattgccaggccagtgagagtgtttataatagcgactggttagcctggtatcagcagaaaccagggcagcctcccaagcaactgatctatgctgcatccactctggcatctggggtcccatcgcgcttcaaaggcagtggatctgggacacagttcactctcaccatcagcgatgtggtgtgtgacgatgctgccacttattattgtgcaggatataaaagtagtagtactgatgggattgctttcggcggagggaccgaggtggtggtcaa

SEQ ID NO: 18 - protein, 134 aa, Artificial Sequence
  Description of Artificial Sequence: Synthetic polypeptide
MDTRAPTQLLGLLLLWLPGATLAIVVTQTPSSKSVPVGGTVTINCQASESVYNSDWLAWYQQKPGQPPKQLIYAASTLASGVPSRFKGSGSGTQFTLTISDVVCDDAATYYCAGYKSSSTDGIAFGGGTEVVVK

SEQ ID NO: 19 - protein, 238 aa, Artificial Sequence
  Description of Artificial Sequence: Synthetic polypeptide
MDTRAPTQLLGLLLLWLPGATLAIVVTQTPSSKSVPVGGTVTINCQASESVYNSDWLAWYQQKPGQPPKQLIYAASTLASGVPSRFKGSGSGTQFTLTISDVVCDDAATYYCAGYKSSSTDGIAFGGGTEVVVKGDPVAPTVLIFPPAADQVATGTVTIVCVANKYFPDVTVTWEVDGTTQTTGIENSKTPQNSADCTYNLSSTLTLTSTQYNSHKEYTCKVTQGTTSVVQSFNRGDC

SEQ ID NO: 20 - DNA, 414 bp, Artificial Sequence
  Description of Artificial Sequence: Synthetic polynucleotide
atggagactgggctgcgctggcttctcctggtcgctgtgctcaaaggtgtccagtgtcaggagcagctggaggagtccgggggaggcctggtcaagcctggggcatccctgacactcacctgcaaagcctctggattcgacttcagtatcaactactacatgtgctgggtccgccaggctccagggaaggggttggagtggatcgcatgcatttatactggtgatgatgacactttctacgcgagctgggcgaaaggccggttcaccatctccaaaacctcgtcgaccacggtgactctacaactgaacagtctgacagccgcggacacggccacctatttctgtgtgagaggtctatatagtggtagtattaataacctgtggggcccaggcaccctggtcaccgtctcctca

SEQ ID NO: 21 - protein, 138 aa, Artificial Sequence
  Description of Artificial Sequence: Synthetic polypeptide
METGLRWLLLVAVLKGVQCQEQLEESGGGLVKPGASLTLTCKASGFDFSINYYMCWVRQAPGKGLEWIACIYTGDDDTFYASWAKGRFTISKTSSTTVTLQLNSLTAADTATYFCVRGLYSGSINNLWGPGTLVTVSS

SEQ ID NO: 22 - protein, 461 aa, Artificial Sequence
  Description of Artificial Sequence: Synthetic polypeptide
METGLRWLLLVAVLKGVQCQEQLEESGGGLVKPGASLTLTCKASGFDFSINYYMCWVRQAPGKGLEWIACIYTGDDDTFYASWAKGRFTISKTSSTTVTLQLNSLTAADTATYFCVRGLYSGSINNLWGPGTLVTVSSGQPKAPSVFPLAPCCGDTPSSTVTLGCLVKGYLPEPVTVTWNSGTLTNGVRTFPSVRQSSGLYSLSSVVSVTSSSQPVTCNVAHPATNTKVDKTVAPSTCSKPTCPPPELLGGPSVFIFPPKPKDTLMISRTPEVTCVVVDVSQDDPEVQFTWYINNEQVRTARPPLREQQFNSTIRVVSTLPIAHQDWLRGKEFKCKVHNKALPAPIEKTISKARGQPLEPKVYTMGPPREELSSRSVSLTCMINGFYPSDISVEWEKNGKAEDNYKTTPAVLDSDGSYFLYSKLSVPTSEWQRGDVFTCSVMHEALHNHYTQKSISRSPGK

SEQ ID NO: 23 - protein, 8 aa, Artificial Sequence
  Description of Artificial Sequence: Synthetic peptide
GFDFSINY

SEQ ID NO: 24 - protein, 5 aa, Artificial Sequence
  Description of Artificial Sequence: Synthetic peptide
YTGDD

SEQ ID NO: 25 - protein, 10 aa, Artificial Sequence
  Description of Artificial Sequence: Synthetic peptide
GLYSGSINNL

SEQ ID NO: 26 - DNA, 402 bp, Artificial Sequence
  Description of Artificial Sequence: Synthetic polynucleotide
atggacacgagggcccccactcagctgctggggctcctgctgctctggctcccagatgccagatgtgcgcttgtgatgacccagactccatcccctgtgtctgcagctgtgggaggcacagtcaccatcagttgccaggccagtcagagtgtttataacaacgactacttatcctggtatcagcagaaaccagggcagcctcccaaactcctgatctattatgcatccactctggcatctggggtctcatcgcggttcaaaggcagtggatctgggacacagttcactctcaccatcagcgacgtgcagtgtgacgatgctgccgcttactattgtgcaggcgttaaaggttatagtaatgataataatggtttcggcggagggaccgaggtggtggtcaaa

SEQ ID NO: 27 - protein, 134 aa, Artificial Sequence
  Description of Artificial Sequence: Synthetic polypeptide
MDTRAPTQLLGLLLLWLPDARCALVMTQTPSPVSAAVGGTVTISCQASQSVYNNDYLSWYQQKPGQPPKLLIYYASTLASGVSSRFKGSGSGTQFTLTISDVQCDDAAAYYCAGVKGYSNDNNGFGGGTEVVVK

SEQ ID NO: 28 - protein, 238 aa, Artificial Sequence
  Description of Artificial Sequence: Synthetic polypeptide
MDTRAPTQLLGLLLLWLPDARCALVMTQTPSPVSAAVGGTVTISCQASQSVYNNDYLSWYQQKPGQPPKLLIYYASTLASGVSSRFKGSGSGTQFTLTISDVQCDDAAAYYCAGVKGYSNDNNGFGGGTEVVVKGDPVAPTVLIFPPAADQVATGTVTIVCVANKYFPDVTVTWEVDGTTQTTGIENSKTPQNSADCTYNLSSTLTLTSTQYNSHKEYTCKVTQGTTSVVQSFNRGDC

SEQ ID NO: 29 - protein, 13 aa, Artificial Sequence
  Description of Artificial Sequence: Synthetic peptide
QASQSVYNNDYLS

SEQ ID NO: 30 - protein, 7 aa, Artificial Sequence
  Description of Artificial Sequence: Synthetic peptide
YASTLAS

SEQ ID NO: 31 - protein, 12 aa, Artificial Sequence
  Description of Artificial Sequence: Synthetic peptide
AGVKGYSNDNNG

SEQ ID NO: 32 - DNA, 411 bp, Artificial Sequence
  Description of Artificial Sequence: Synthetic polynucleotide
atggagactgggctgcgctggcttctcctggtcgctgtgctcaaaggtgtccaatgtcagtcgctggaggagtccgggggaggcctggtcaagcctggggcatccctgacactcacctgcaaagcctctggattcgacttcagtatcaactactacatgtgctgggtccgccaggctccagggaaggggttggagtggatcgcatgcatttatactggtgatgatgacactttctacgcgagctgggcgaaaggccggttcaccatctccaaaacctcgtcgaccacggtgactctacaactgaacagtctgacagccgcggacacggccacctatttctgtgtgagaggtctatatagtggtagtattaataacctgtggggcccaggcaccctggtcaccgtctcctca

SEQ ID NO: 33 - protein, 137 aa, Artificial Sequence
  Description of Artificial Sequence: Synthetic polypeptide
METGLRWLLLVAVLKGVQCQSLEESGGGLVKPGASLTLTCKASGFDFSINYYMCWVRQAPGKGLEWIACIYTGDDDTFYASWAKGRFTISKTSSTTVTLQLNSLTAADTATYFCVRGLYSGSINNLWGPGTLVTVSS

SEQ ID NO: 34 - protein, 460 aa, Artificial Sequence
  Description of Artificial Sequence: Synthetic polypeptide
METGLRWLLLVAVLKGVQCQSLEESGGGLVKPGASLTLTCKASGFDFSINYYMCWVRQAPGKGLEWIACIYTGDDDTFYASWAKGRFTISKTSSTTVTLQLNSLTAADTATYFCVRGLYSGSINNLWGPGTLVTVSSGQPKAPSVFPLAPCCGDTPSSTVTLGCLVKGYLPEPVTVTWNSGTLTNGVRTFPSVRQSSGLYSLSSVVSVTSSSQPVTCNVAHPATNTKVDKTVAPSTCSKPTCPPPELLGGPSVFIFPPKPKDTLMISRTPEVTCVVVDVSQDDPEVQFTWYINNEQVRTARPPLREQQFNSTIRVVSTLPIAHQDWLRGKEFKCKVHNKALPAPIEKTISKARGQPLEPKVYTMGPPREELSSRSVSLTCMINGFYPSDISVEWEKNGKAEDNYKTTPAVLDSDGSYFLYSKLSVPTSEWQRGDVFTCSVMHEALHNHYTQKSISRSPGK

SEQ ID NO: 35 - DNA, 402 bp, Artificial Sequence; identical to SEQ ID NO: 26
  Description of Artificial Sequence: Synthetic polynucleotide

SEQ ID NO: 36 - protein, 134 aa, Artificial Sequence; identical to SEQ ID NO: 27
  Description of Artificial Sequence: Synthetic polypeptide

SEQ ID NO: 37 - protein, 238 aa, Artificial Sequence; identical to SEQ ID NO: 28
  Description of Artificial Sequence: Synthetic polypeptide

SEQ ID NO: 38 - DNA, 417 bp, Artificial Sequence
  Description of Artificial Sequence: Synthetic polynucleotide
atggagactgggctgcgctggcttctcctggtcgctgtgctcaaaggggtccagtgtcagtcgttggaggagtccgggggagacctggtcaagcctggggcatccctgacactcacctgcacagcctctggattctccttcacgagcaactactacatgtgctgggtccgccaggctccagggaaggggctggagtgggtcgcgtgcatttttcttggtagtagtggtaacactgtctacgcgaactgggcgaaaggccgattcaccatctccaaaacctcgtcgaccacggtgactctgcaaatgaccagtctgacagtcgcggacacggccacctatttctgtgcgagagactatgttaatggttatgactactttaacttgtggggcccaggcaccttggtcaccgtctcctca

SEQ ID NO: 39 - protein, 139 aa, Artificial Sequence
  Description of Artificial Sequence: Synthetic polypeptide
METGLRWLLLVAVLKGVQCQSLEESGGDLVKPGASLTLTCTASGFSFTSNYYMCWVRQAPGKGLEWVACIFLGSSGNTVYANWAKGRFTISKTSSTTVTLQMTSLTVADTATYFCARDYVNGYDYFNLWGPGTLVTVSS

SEQ ID NO: 40 - protein, 462 aa, Artificial Sequence
  Description of Artificial Sequence: Synthetic polypeptide
METGLRWLLLVAVLKGVQCQSLEESGGDLVKPGASLTLTCTASGFSFTSNYYMCWVRQAPGKGLEWVACIFLGSSGNTVYANWAKGRFTISKTSSTTVTLQMTSLTVADTATYFCARDYVNGYDYFNLWGPGTLVTVSSGQPKAPSVFPLAPCCGDTPSSTVTLGCLVKGYLPEPVTVTWNSGTLTNGVRTFPSVRQSSGLYSLSSVVSVTSSSQPVTCNVAHPATNTKVDKTVAPSTCSKPTCPPPELLGGPSVFIFPPKPKDTLMISRTPEVTCVVVDVSQDDPEVQFTWYINNEQVRTARPPLREQQFNSTIRVVSTLPIAHQDWLRGKEFKCKVHNKALPAPIEKTISKARGQPLEPKVYTMGPPREELSSRSVSLTCMINGFYPSDISVEWEKNGKAEDNYKTTPAVLDSDGSYFLYSKLSVPTSEWQRGDVFTCSVMHEALHNHYTQKSISRSPGK

SEQ ID NO: 41 - protein, 8 aa, Artificial Sequence
  Description of Artificial Sequence: Synthetic peptide
GFSFTSNY

SEQ ID NO: 42 - protein, 6 aa, Artificial Sequence
  Description of Artificial Sequence: Synthetic peptide
FLGSSG

SEQ ID NO: 43 - protein, 11 aa, Artificial Sequence
  Description of Artificial Sequence: Synthetic peptide
DYVNGYDYFNL

SEQ ID NO: 44 - DNA, 402 bp, Artificial Sequence
  Description of Artificial Sequence: Synthetic polynucleotide
atggacacgagggcccccactcagctgctggggctcctgctgctctggctcccaggtgccacatttgcccaagtgctgacccagactgcatcccccgtgtctgcggctgttggaggcacagtcaccatcaattgccagtccagtcagagtgtttataataagaacttagcctggtatcagcagaaaccagggcagcctcccaaaggcctgatctattctacatcgactctagattctggggtcccatcgcggttcagcggcagtggatctgggacacagttcactctcaccatcagcgacgtgcagtgtgacgatgctgccacttactactgtctaggcagttatgattgtagtagtgctgattgtaatgctttcggcggagggaccgaggtggtggtcaaa

SEQ ID NO: 45 - protein, 134 aa, Artificial Sequence
  Description of Artificial Sequence: Synthetic polypeptide
MDTRAPTQLLGLLLLWLPGATFAQVLTQTASPVSAAVGGTVTINCQSSQSVYNKNLAWYQQKPGQPPKGLIYSTSTLDSGVPSRFSGSGSGTQFTLTISDVQCDDAATYYCLGSYDCSSADCNAFGGGTEVVVK

SEQ ID NO: 46 - protein, 238 aa, Artificial Sequence
  Description of Artificial Sequence: Synthetic polypeptide
MDTRAPTQLLGLLLLWLPGATFAQVLTQTASPVSAAVGGTVTINCQSSQSVYNKNLAWYQQKPGQPPKGLIYSTSTLDSGVPSRFSGSGSGTQFTLTISDVQCDDAATYYCLGSYDCSSADCNAFGGGTEVVVKGDPVAPTVLIFPPAADQVATGTVTIVCVANKYFPDVTVTWEVDGTTQTTGIENSKTPQNSADCTYNLSSTLTLTSTQYNSHKEYTCKVTQGTTSVVQSFNRGDC

SEQ ID NO: 47 - protein, 12 aa, Artificial Sequence
  Description of Artificial Sequence: Synthetic peptide
QSSQSVYNKNLA

SEQ ID NO: 48 - protein, 7 aa, Artificial Sequence
  Description of Artificial Sequence: Synthetic peptide
STSTLDS

SEQ ID NO: 49 - protein, 13 aa, Artificial Sequence
  Description of Artificial Sequence: Synthetic peptide
LGSYDCSSADCNA

SEQ ID NO: 50 - DNA, 399 bp, Artificial Sequence
  Description of Artificial Sequence: Synthetic polynucleotide
atggagactgggctgcgctggcttctcctggtcgctgtgctcaaaggtgtccaatgtcagtcgctggaggagtccgggggaggcctggtcaagcctggggcatccctgacactcacctgcacagcctctggattctccttcagtgacagttggtacttgtgttgggtccgccaggctccagggaaggggctggagtggatcgcatgcatttatactggtgatggtgacacttattacgcgacctgggcgaaaggccgattcaccatctccaagacctcgtcgaccacagtgactctacaaatgaccagtctgacagccgcggacacggccacctatttctgtgcgaggggtgcccaattttacttgtggggccaaggcaccctggtcaccgtctcctca

SEQ ID NO: 51 - protein, 133 aa, Artificial Sequence
  Description of Artificial Sequence: Synthetic polypeptide
METGLRWLLLVAVLKGVQCQSLEESGGGLVKPGASLTLTCTASGFSFSDSWYLCWVRQAPGKGLEWIACIYTGDGDTYYATWAKGRFTISKTSSTTVTLQMTSLTAADTATYFCARGAQFYLWGQGTLVTVSS

SEQ ID NO: 52 - protein, 456 aa, Artificial Sequence
  Description of Artificial Sequence: Synthetic polypeptide
METGLRWLLLVAVLKGVQCQSLEESGGGLVKPGASLTLTCTASGFSFSDSWYLCWVRQAPGKGLEWIACIYTGDGDTYYATWAKGRFTISKTSSTTVTLQMTSLTAADTATYFCARGAQFYLWGQGTLVTVSSGQPKAPSVFPLAPCCGDTPSSTVTLGCLVKGYLPEPVTVTWNSGTLTNGVRTFPSVRQSSGLYSLSSVVSVTSSSQPVTCNVAHPATNTKVDKTVAPSTCSKPTCPPPELLGGPSVFIFPPKPKDTLMISRTPEVTCVVVDVSQDDPEVQFTWYINNEQVRTARPPLREQQFNSTIRVVSTLPIAHQDWLRGKEFKCKVHNKALPAPIEKTISKARGQPLEPKVYTMGPPREELSSRSVSLTCMINGFYPSDISVEWEKNGKAEDNYKTTPAVLDSDGSYFLYSKLSVPTSEWQRGDVFTCSVMHEALHNHYTQKSISRSPGK

SEQ ID NO: 53 - protein, 8 aa, Artificial Sequence
  Description of Artificial Sequence: Synthetic peptide
GFSFSDSW

SEQ ID NO: 54 - protein, 5 aa, Artificial Sequence
  Description of Artificial Sequence: Synthetic peptide
YTGDG

SEQ ID NO: 55 - protein, 6 aa, Artificial Sequence
  Description of Artificial Sequence: Synthetic peptide
GAQFYL

SEQ ID NO: 56 - DNA, 405 bp, Artificial Sequence
  Description of Artificial Sequence: Synthetic polynucleotide
atggacacgagggcccccactcagctgctggggctcctgctgctctggctcccaggtgccacatttgcccaggtgctgacccagactccatcctccgtgtctgcagctgtgggaggcacagtcaccatcaattgccagtccagtcagagtgtttatgccaacacctacttatcctggtatcagcagaaaccagggcagcctcccaagcaactgatctattctgcatccagtctggcatctggggtcccaccgcggttcaaaggcagtggatctgggacacagttcgctctcaccatcagcgacgtgcagtgtgacgatgctgccacttactactgtctaggcagatatagttgtggtcttgctgattgtgctgctttcggcggagggaccgaggtggtggtcaaa

SEQ ID NO: 57 - protein, 135 aa, Artificial Sequence
  Description of Artificial Sequence: Synthetic polypeptide
MDTRAPTQLLGLLLLWLPGATFAQVLTQTPSSVSAAVGGTVTINCQSSQSVYANTYLSWYQQKPGQPPKQLIYSASSLASGVPPRFKGSGSGTQFALTISDVQCDDAATYYCLGRYSCGLADCAAFGGGTEVVVK

SEQ ID NO: 58 - protein, 239 aa, Artificial Sequence
  Description of Artificial Sequence: Synthetic polypeptide
MDTRAPTQLLGLLLLWLPGATFAQVLTQTPSSVSAAVGGTVTINCQSSQSVYANTYLSWYQQKPGQPPKQLIYSASSLASGVPPRFKGSGSGTQFALTISDVQCDDAATYYCLGRYSCGLADCAAFGGGTEVVVKGDPVAPTVLIFPPAADQVATGTVTIVCVANKYFPDVTVTWEVDGTTQTTGIENSKTPQNSADCTYNLSSTLTLTSTQYNSHKEYTCKVTQGTTSVVQSFNRGDC

SEQ ID NO: 59 - protein, 13 aa, Artificial Sequence
  Description of Artificial Sequence: Synthetic peptide
QSSQSVYANTYLS

SEQ ID NO: 60 - protein, 7 aa, Artificial Sequence
  Description of Artificial Sequence: Synthetic peptide
SASSLAS

SEQ ID NO: 61 - protein, 13 aa, Artificial Sequence
  Description of Artificial Sequence: Synthetic peptide
LGRYSCGLADCAA

SEQ ID NO: 62 - protein, 5 aa, Artificial Sequence
  Description of Artificial Sequence: Synthetic peptide
NNGIC

SEQ ID NO: 63 - protein, 17 aa, Artificial Sequence
  Description of Artificial Sequence: Synthetic peptide
CLYVGSSDTTYYASWAK

SEQ ID NO: 64 - protein, 6 aa, Artificial Sequence
  Description of Artificial Sequence: Synthetic peptide
INYYMC

SEQ ID NO: 65 - protein, 16 aa, Artificial Sequence
  Description of Artificial Sequence: Synthetic peptide
CIYTGDDDTFYASWAK

SEQ ID NO: 66 - protein, 6 aa, Artificial Sequence
  Description of Artificial Sequence: Synthetic peptide
SNYYMC

SEQ ID NO: 67 - protein, 17 aa, Artificial Sequence
  Description of Artificial Sequence: Synthetic peptide
CIFLGSSGNTVYANWAK

SEQ ID NO: 68 - protein, 6 aa, Artificial Sequence
  Description of Artificial Sequence: Synthetic peptide
DSWYLC

SEQ ID NO: 69 - protein, 16 aa, Artificial Sequence
  Description of Artificial Sequence: Synthetic peptide
CIYTGDGDTYYATWAK

SEQ ID NO: 70 - protein, 10 aa, Artificial Sequence
  Description of Artificial Sequence: Synthetic peptide
GFSFSNNGIC

SEQ ID NO: 71 - protein, 11 aa, Artificial Sequence
  Description of Artificial Sequence: Synthetic peptide
GFDFSINYYMC

SEQ ID NO: 72 - protein, 11 aa, Artificial Sequence
  Description of Artificial Sequence: Synthetic peptide
GFSFTSNYYMC

SEQ ID NO: 73 - protein, 11 aa, Artificial Sequence
  Description of Artificial Sequence: Synthetic peptide
GFSFSDSWYLC

SEQ ID NO: 74 - protein, 11 aa, Artificial Sequence
  Synthetic polypeptide
RASQDISKYLN

SEQ ID NO: 75 - protein, 7 aa, Artificial Sequence
  Synthetic polypeptide
HTSRLHS

SEQ ID NO: 76 - protein, 9 aa, Artificial Sequence
  Synthetic polypeptide
QQGNTLPYT

SEQ ID NO: 77 - protein, 7 aa, Artificial Sequence
  Synthetic polypeptide
GVSLPDY

SEQ ID NO: 78 - protein, 5 aa, Artificial Sequence
  Synthetic polypeptide
WGSET

SEQ ID NO: 79 - protein, 12 aa, Artificial Sequence
  Synthetic polypeptide
HYYYGGSYAMDY

SEQ ID NO: 80 - protein, 5 aa, Artificial Sequence
  Synthetic polypeptide
DYGVS

SEQ ID NO: 81 - protein, 16 aa, Artificial Sequence
  Synthetic polypeptide
VIWGSETTYYNSALKS

SEQ ID NO: 82 - protein, 10 aa, Artificial Sequence
  Synthetic polypeptide
GVSLPDYGVS